European Patent Application EP 4 800 027 A1, published September 2, 2026. Title: 一种VIPR1L蛋白及其在生物农药及生物育种上的应用. Applicant: 北京中农阿拉丁生物科技有限责任公司. The sequence listing filed with the application follows.

SEQUENCE LISTING (217 sequences)

SEQ ID NO: 1 - protein, 130 aa, Gossypium barbadense
MIPQQMKEAFQSYIAFKSDSSPFSRMAKSTPALSEFDNYHKAKVSSLEEPSKSKSKTIKELVTMSSKLDSLEKGESFLREKIQAQKLKYNDKPDSLRQSNGEAFQKYLEDTTKNLIKAMPNLKANLVLHA

SEQ ID NO: 2 - DNA, 393 bp, Gossypium barbadense
  source 1..393: mol_type = other DNA
atgatccctcaacaaatgaaagaggccttccaatcttacattgcattcaagtcagactcatctcctttttcacggatggctaaatctaccccggctctatcagagttcgacaactaccataaagccaaggtttctagcttggaggagccaagtaaatcaaaaagcaagacgataaaggagttagttacaatgagcagtaagcttgattcattggagaaaggcgagtccttcttaagggaaaaaatccaagcccagaagctaaaatataatgacaagccggatagccttcgccagtccaatggtgaagcctttcaaaagtacctagaggacacaaccaagaacttgatcaaggcaatgccaaatctaaaggctaacttggtccttcatgcctaa

SEQ ID NO: 3 - protein, 297 aa, Verticillium dahliae
MLSLQTAALLLFPLVAASPVARAAETSVTVTVDTAPAGPTSSTYNWAEGWKANFPIHQSCNITLRTQLEAALAETMTIAAHARDHLLHNPKSELATKFFGNQSVAGPIGWYSKVVSTDKSEMLFRCDDPDRNCATQDGWAGHWRGSNATQETVICDLSYEIRRPLAALCGGGYTVAESKLNTYWATDLLHRAFHLPGISDGIIDHYAEDYAEALKLAATEPELSIIDSDTLQYFAIEAYAYDIAIPGVGCPGEKPIIDTAAGTSTAAPTTTTASDASGTTTANASCHTHDDGFVHCS

SEQ ID NO: 4 - DNA, 894 bp, Verticillium dahliae
  source 1..894: mol_type = other DNA
atgctttctctccagaccgcagccctgctgctcttccctctcgtcgctgcctctcccgtggcacgcgctgctgagaccagtgttaccgtcacggtggacactgcccctgccggccctaccagctccacctacaactgggccgaaggctggaaggccaacttccccatccaccagtcttgcaacatcacccttcgtactcagctcgaggctgctctcgccgagaccatgaccattgcggcccacgcccgcgatcatcttctccacaaccccaagtccgagctggcgacgaagttcttcggcaaccagtctgtcgccggccccatcggctggtactccaaggtcgtctcgaccgacaagtctgagatgctcttccgctgcgacgaccctgatcgtaactgcgctacccaagatggctgggccggccactggcgcggctcgaatgccacccaggagacggtcatctgcgacctctcctacgagatccgccgccctcttgccgctctctgcggtggtggttataccgtggccgagtccaagctcaacacctactgggccactgaccttctgcaccgcgccttccacctgcccggcatcagcgacggcatcatcgatcactacgctgaggattacgccgaggccctcaagcttgccgccactgagcctgaactctccatcatcgacagcgacacccttcagtacttcgccattgaggcttatgcctatgacattgccatccccggcgtcggctgccccggcgagaagcccatcattgacaccgccgccggcaccagcaccgctgccccgactactactaccgccagcgatgccagcggcaccaccaccgccaatgcttcgtgccacacccacgacgatggctttgttcactgctcgtag

SEQ ID NO: 5 - DNA, 1968 bp, Lachnellula hyalina
  source 1..1968: mol_type = other DNA
atgctcacccagttttttttcattgccattctttcttcactcctactgcaggtggccaaaccagatcttgtcaccgacagagcttctcttttgagccttcgttcctcagtcggaggcagaaccctcttatggaacgtctcgaaccagagtccatgctcgtgggctggggttacgtgcgagcggaaccgcgtcacagtgcttagactacctggtgttgctctctctggccaaattccgactggcattttcgggaacttgactcagctgcgcaccctcagtctacgtcttaactcgttaactggaccactcccttcggatcttgctctctgtcaaaacctccgaaacctttacttgcagggaaaccatttttcgggtgagataccggaattcctgtttggtcttcatgatttagtgaggctaagtctttctgggaacaacttttctggggaagtctctgttgggttcaacaatttgacgaggttgagaactttgcttcttgacagcaatagtctttctgggtcggtacctgagttgggttctttgcaaaaccttggccaatttaatgtgtcaaataatttgttgaacggctcaatccccaaggggttacagaaatatgggtccgatgcttttctggggaatttgctttgtgggaaaccacttgacaaggcttgccctgccactgctactgctgctcctgggaatacaagtgagcccgccaatccaacgaatgagaataaaccagagaaaaagaagaagagcaagttgtctgggggtgcaattgcaggtattgttattggatctgtgctcggatttcttctgattgttgtgattttaatgattttatgtagaaagaagagtagcaagcaatcgaggtcaattgacatcacttcgcttaagaatcaagaaatggagattcctggggagaaatcaggtggggaaatggagaatggtggatatgcgaatgggaatgggaatgggtattcagtggcagcggcggcagtagcagcaatggtgggtggtggagccaaagcggcggaaaacagtgggaccggagctaagaagttggtcttctttgggaatgcaacgcgagtgtttgatttggaggatttgttgagagcttctgcagaggttttaggtaaaggcacgtttggaacagcatataaagcagtgttggaaggtggaaacgcagtggctgttaagagactcaaggatgtcactatatctgagagggaatttaaggataagatcgaaggggttggagctatggatcatcagcatttggtccctctcagagcttactattttagtagggatgagaagcttcttgtttatgattacatgcccatgggaagcttatcagcgcttttgcatgggaataaaggggcaggaaggactccactgaactgggacattaggtctggaattgctcttggagctgcctgtggaattgaatacctccactctcaaggccctaatgtctctcatggaaacataaaatcttcaaatatcctcctcactaaatcctatgaagctcgagtttcggattttggactggcaaacattgtaggttcatcgtccagtcccaatagagtgctggggtaccgggcaccagaggtgactgacccccgcaaagtatcacaaaaggctgatgtttatagctttggtgtgttgcttttggagttattgactgggaaagcccccacccattcaatcttgaacgaggaaggaattgacctcccgaggtgggtgcagtctgttgttcgtgaagaatggacttccgaggtgtttgatcttgagctcctcaggtatcagaatgtggaggaagagatggtccaactcttgcaacttgctgttgattgtgctgcacaataccctgacaagcgccccaccatgtctcaagtgaggagccgaatcgaggagctacgtcaatctagtttgcgagacgatctgatcccacagtctgcctga

SEQ ID NO: 6 - protein, 130 aa, Gossypium barbadense
MIPQQKKKKKQSYFKIASDSSAAQQMAKSTNYHPALSEFDKVKVLEESSPSKSKSKTIKELVTMSSKLDSLEKGESFLREKIQAQKLKYNDKPDSLRQSNGEAFQKYLEDTTKNLIKAMPAQQANLVLHA

SEQ ID NO: 7 - protein, 130 aa, Gossypium barbadense
QQMMIPKEAFFKSDSQSYIASPFSRMKASTPALLEFDYYHKVKVSALEEPSKSKSKTIKELVTMSSKLDSLEKGESFLREKIQAQKLKYNDKPDSLRQSNGEAFQKYLEDTTKNLIKAMPNLAKNLVLHA

SEQ ID NO: 8 - protein, 130 aa, Gossypium barbadense
MIPQQMVEAFQSYLAFKSDSSPFSSMAKSTPALSFEDNYHSSLEKAKVEPSKSKSKTIKELVTMSSKLDSLEKGESFLREKIQAQKLKYNDKPDSLRQSNGEAFQKYLEDTTKNLIKAMPNLKANLLVHA

SEQ ID NO: 9 - protein, 130 aa, Gossypium barbadense
MIPQQMKEAFQSYIAFKSDSMAKSTSPFSRPALSEFDNYHKAKVSSLFEPSKSKSKTIKELVTMSSKLDSLEKGESFLREKIQAQKLKYNDKPDSLRQSNGEAFQKYLEDTTKNLIKAMPNLKANLVLHA

SEQ ID NO: 10 - protein, 130 aa, Gossypium barbadense
MIPQPMKEAFQSYIAFKSDSSPFSVMAKSTPALSEFDNYHKAKVSALEEPSKSKSKTIKELVTMSSKLDSLEKGESFLREKIQAQKLKYNDKPDSLRQSNGEAFQKYLEDTTKNLIKAMPNLKAMLVLHA

SEQ ID NO: 11 - protein, 130 aa, Gossypium barbadense
MPPQAMKLFFQSVIAKKSLSSPVSSSATSTPAISGFDNMIKAKASSLEEPSKEKSKTIKQIVTMSSKLMSLEKGESQLRVKLRMQKLKYNKKKDSLRQSNPEAFQKYLEDTTKNVIKMQVNRKANLVLHA

SEQ ID NO: 12 - protein, 130 aa, Gossypium barbadense
MPPQQMKLFFQSVIAFKSLSSPVSRMATSTPAISGFDNMIKAKASSLEEPSKEKSKTIKQIVTMSSKLMSLEKGESFLRVKLRMQKLKYNDKPDSLRQSNGEAFQKYLEDTTKNVIKMQVNRKANLVLHA

SEQ ID NO: 13 - protein, 130 aa, Gossypium barbadense
MIPQLMKGMFQSYIMFTSDDSPFSRMAVSTPALVEFDNYKKAKVSSLVSPSKSKSKTIKEVVTRSSKLDSLEKGESLLREKRQSQKLKYNDKPDSLRQSNGEAFQKYLEDTTKNLMKAMRVLKANLVLHA

SEQ ID NO: 14 - protein, 130 aa, Gossypium barbadense
MIPQLMKKMFQSYIMFKSDSSPFSRMAVSTPALVEFDNYKKAKVSSLESPSKSKSKTIKEVVTRSSKLDSLEKGESFLREKRQSQKLKYNDKPDSLRQSNGEAFQKYLEDTTKNLMKAMRVLKANLVLHA

SEQ ID NO: 15 - protein, 130 aa, Gossypium barbadense
MIPQQMKLAFQSYIAFKSDSSPFSRMATSTPALSEFDNYHKAKVSSLEEPSKEKSKTIKELVTMSSKLDSLEKGESFLREKIRAQKLKYNDKPDSLRQSNGEAFQKYLEDTTKNLIKAQPNLKANLVLHA

SEQ ID NO: 16 - protein, 135 aa, Gossypium barbadense
MIPQQMKEAFQSYIAFKSDSSPFSRMAKSTPALSEFDNYHKAKVSSLEEPSKSKSPTIKELVTPSSKLDSLEKGESFLREKIQAQKKKYNDKPASLPQSNGEAFQKYLEDTTKNLIKAMPNLKANLVLHARRRRR

SEQ ID NO: 17 - protein, 135 aa, Gossypium barbadense
RRRRRMIPQQMKEAFQSYIAFKSDSSPFSRMAKSTPALSEFDNYHKAKVSSLEEPSKSKSPTIKELVTPSSKLDSLEKGESFLREKIQAQKKKYNDKPASLPQSNGEAFQKYLEDTTKNLIKAMPNLKANLVLHA

SEQ ID NO: 18 - protein, 136 aa, Gossypium barbadense
MIPQQMKEAFQSYIAFKSDSSPFSRMAKSTPALSEFDNYHKAKVSSLEEPSKSKSPTIKELVTPSSKLDSLEKGESFLREKIQAQKKKYNDKPASLPQSNGEAFQKYLEDTTKNLIKAMPNLKANLVLHARRRRRR

SEQ ID NO: 19 - protein, 136 aa, Gossypium barbadense
RRRRRRMIPQQMKEAFQSYIAFKSDSSPFSRMAKSTPALSEFDNYHKAKVSSLEEPSKSKSPTIKELVTPSSKLDSLEKGESFLREKIQAQKKKYNDKPASLPQSNGEAFQKYLEDTTKNLIKAMPNLKANLVLHA

SEQ ID NO: 20 - protein, 132 aa, Gossypium barbadense
MIPQQMKEAFQSYIAFKSDSSPFSRMAKSTPALSEFDNYHKAKVSSLEEPSKSKSPTIKELVTPSSKLDSLEKGESFLREKIQAQKKKYNDKPASLPQSNGEAFQKYLEDTTKNLIKAMPNLKANLVLHAHH

SEQ ID NO: 21 - protein, 140 aa, Gossypium barbadense
HHHHHHHHHHMIPQQMKEAFQSYIAFKSDSSPFSRMAKSTPALSEFDNYHKAKVSSLEEPSKSKSPTIKELVTPSSKLDSLEKGESFLREKIQAQKKKYNDKPASLPQSNGEAFQKYLEDTTKNLIKAMPNLKANLVLHA

SEQ ID NO: 22 - protein, 134 aa, Gossypium barbadense
MIPQQMKEAFQSYIAFKSDSSPFSRMAKSTPALSEFDNYHKAKVSSLEEPSKSKSPTIKELVTPSSKLDSLEKGESFLREKIQAQKKKYNDKPASLPQSNGEAFQKYLEDTTKNLIKAMPNLKANLVLHAHHHH

SEQ ID NO: 23 - protein, 132 aa, Gossypium barbadense
HHMIPQQMKEAFQSYIAFKSDSSPFSRMAKSTPALSEFDNYHKAKVSSLEEPSKSKSPTIKELVTPSSKLDSLEKGESFLREKIQAQKKKYNDKPASLPQSNGEAFQKYLEDTTKNLIKAMPNLKANLVLHA

SEQ ID NO: 24 - protein, 137 aa, Gossypium barbadense
HHHHHHHMIPQQMKEAFQSYIAFKSDSSPFSRMAKSTPALSEFDNYHKAKVSSLEEPSKSKSPTIKELVTPSSKLDSLEKGESFLREKIQAQKKKYNDKPASLPQSNGEAFQKYLEDTTKNLIKAMPNLKANLVLHA

SEQ ID NO: 25 - protein, 140 aa, Gossypium barbadense
MIPQQMKEAFQSYIAFKSDSSPFSRMAKSTPALSEFDNYHKAKVSSLEEPSKSKSPTIKELVTPSSKLDSLEKGESFLREKIQAQKKKYNDKPASLPQSNGEAFQKYLEDTTKNLIKAMPNLKANLVLHAHHHHHHHHHH

SEQ ID NO: 26 - protein, 138 aa, Gossypium barbadense
MIPQQMKEAFQSYIAFKSDSSPFSRMAKSTPALSEFDNYHKAKVSSLEEPSKSKSPTIKELVTPSSKLDSLEKGESFLREKIQAQKKKYNDKPASLPQSNGEAFQKYLEDTTKNLIKAMPNLKANLVLHADYKDDDDK

SEQ ID NO: 27 - protein, 138 aa, Gossypium barbadense
DYKDDDDKMIPQQMKEAFQSYIAFKSDSSPFSRMAKSTPALSEFDNYHKAKVSSLEEPSKSKSPTIKELVTPSSKLDSLEKGESFLREKIQAQKKKYNDKPASLPQSNGEAFQKYLEDTTKNLIKAMPNLKANLVLHA

SEQ ID NO: 28 - protein, 138 aa, Gossypium barbadense
MIPQQMKEAFQSYIAFKSDSSPFSRMAKSTPALSEFDNYHKAKVSSLEEPSKSKSPTIKELVTPSSKLDSLEKGESFLREKIQAQKKKYNDKPASLPQSNGEAFQKYLEDTTKNLIKAMPNLKANLVLHAWSHPQFEK

SEQ ID NO: 29 - protein, 138 aa, Gossypium barbadense
WSHPQFEKMIPQQMKEAFQSYIAFKSDSSPFSRMAKSTPALSEFDNYHKAKVSSLEEPSKSKSPTIKELVTPSSKLDSLEKGESFLREKIQAQKKKYNDKPASLPQSNGEAFQKYLEDTTKNLIKAMPNLKANLVLHA

SEQ ID NO: 30 - protein, 140 aa, Gossypium barbadense
MIPQQMKEAFQSYIAFKSDSSPFSRMAKSTPALSEFDNYHKAKVSSLEEPSKSKSPTIKELVTPSSKLDSLEKGESFLREKIQAQKKKYNDKPASLPQSNGEAFQKYLEDTTKNLIKAMPNLKANLVLHAEQKLISEEDL

SEQ ID NO: 31 - protein, 140 aa, Gossypium barbadense
EQKLISEEDLMIPQQMKEAFQSYIAFKSDSSPFSRMAKSTPALSEFDNYHKAKVSSLEEPSKSKSPTIKELVTPSSKLDSLEKGESFLREKIQAQKKKYNDKPASLPQSNGEAFQKYLEDTTKNLIKAMPNLKANLVLHA

SEQ ID NO: 32 - protein, 135 aa, Gossypium barbadense
MIPQQKKKKKQSYFKIASDSSAAQQMAKSTNYHPALSEFDKVKVLEESSPSKSKSKTIKELVTMSSKLDSLEKGESFLREKIQAQKLKYNDKPDSLRQSNGEAFQKYLEDTTKNLIKAMPAQQANLVLHARRRRR

SEQ ID NO: 33 - protein, 135 aa, Gossypium barbadense
RRRRRMIPQQKKKKKQSYFKIASDSSAAQQMAKSTNYHPALSEFDKVKVLEESSPSKSKSKTIKELVTMSSKLDSLEKGESFLREKIQAQKLKYNDKPDSLRQSNGEAFQKYLEDTTKNLIKAMPAQQANLVLHA

SEQ ID NO: 34 - protein, 136 aa, Gossypium barbadense
MIPQQKKKKKQSYFKIASDSSAAQQMAKSTNYHPALSEFDKVKVLEESSPSKSKSKTIKELVTMSSKLDSLEKGESFLREKIQAQKLKYNDKPDSLRQSNGEAFQKYLEDTTKNLIKAMPAQQANLVLHARRRRRR

SEQ ID NO: 35 - protein, 136 aa, Gossypium barbadense
RRRRRRMIPQQKKKKKQSYFKIASDSSAAQQMAKSTNYHPALSEFDKVKVLEESSPSKSKSKTIKELVTMSSKLDSLEKGESFLREKIQAQKLKYNDKPDSLRQSNGEAFQKYLEDTTKNLIKAMPAQQANLVLHA

SEQ ID NO: 36 - protein, 132 aa, Gossypium barbadense
MIPQQKKKKKQSYFKIASDSSAAQQMAKSTNYHPALSEFDKVKVLEESSPSKSKSKTIKELVTMSSKLDSLEKGESFLREKIQAQKLKYNDKPDSLRQSNGEAFQKYLEDTTKNLIKAMPAQQANLVLHAHH

SEQ ID NO: 37 - protein, 140 aa, Gossypium barbadense
HHHHHHHHHHMIPQQKKKKKQSYFKIASDSSAAQQMAKSTNYHPALSEFDKVKVLEESSPSKSKSKTIKELVTMSSKLDSLEKGESFLREKIQAQKLKYNDKPDSLRQSNGEAFQKYLEDTTKNLIKAMPAQQANLVLHA

SEQ ID NO: 38 - protein, 134 aa, Gossypium barbadense
MIPQQKKKKKQSYFKIASDSSAAQQMAKSTNYHPALSEFDKVKVLEESSPSKSKSKTIKELVTMSSKLDSLEKGESFLREKIQAQKLKYNDKPDSLRQSNGEAFQKYLEDTTKNLIKAMPAQQANLVLHAHHHH

SEQ ID NO: 39 - protein, 132 aa, Gossypium barbadense
HHMIPQQKKKKKQSYFKIASDSSAAQQMAKSTNYHPALSEFDKVKVLEESSPSKSKSKTIKELVTMSSKLDSLEKGESFLREKIQAQKLKYNDKPDSLRQSNGEAFQKYLEDTTKNLIKAMPAQQANLVLHA

SEQ ID NO: 40 - protein, 137 aa, Gossypium barbadense
HHHHHHHMIPQQKKKKKQSYFKIASDSSAAQQMAKSTNYHPALSEFDKVKVLEESSPSKSKSKTIKELVTMSSKLDSLEKGESFLREKIQAQKLKYNDKPDSLRQSNGEAFQKYLEDTTKNLIKAMPAQQANLVLHA

SEQ ID NO: 41 - protein, 140 aa, Gossypium barbadense
MIPQQKKKKKQSYFKIASDSSAAQQMAKSTNYHPALSEFDKVKVLEESSPSKSKSKTIKELVTMSSKLDSLEKGESFLREKIQAQKLKYNDKPDSLRQSNGEAFQKYLEDTTKNLIKAMPAQQANLVLHAHHHHHHHHHH

SEQ ID NO: 42 - protein, 138 aa, Gossypium barbadense
MIPQQKKKKKQSYFKIASDSSAAQQMAKSTNYHPALSEFDKVKVLEESSPSKSKSKTIKELVTMSSKLDSLEKGESFLREKIQAQKLKYNDKPDSLRQSNGEAFQKYLEDTTKNLIKAMPAQQANLVLHADYKDDDDK

SEQ ID NO: 43 - protein, 138 aa, Gossypium barbadense
DYKDDDDKMIPQQKKKKKQSYFKIASDSSAAQQMAKSTNYHPALSEFDKVKVLEESSPSKSKSKTIKELVTMSSKLDSLEKGESFLREKIQAQKLKYNDKPDSLRQSNGEAFQKYLEDTTKNLIKAMPAQQANLVLHA

SEQ ID NO: 44 - protein, 138 aa, Gossypium barbadense
MIPQQKKKKKQSYFKIASDSSAAQQMAKSTNYHPALSEFDKVKVLEESSPSKSKSKTIKELVTMSSKLDSLEKGESFLREKIQAQKLKYNDKPDSLRQSNGEAFQKYLEDTTKNLIKAMPAQQANLVLHAWSHPQFEK

SEQ ID NO: 45 - protein, 138 aa, Gossypium barbadense
WSHPQFEKMIPQQKKKKKQSYFKIASDSSAAQQMAKSTNYHPALSEFDKVKVLEESSPSKSKSKTIKELVTMSSKLDSLEKGESFLREKIQAQKLKYNDKPDSLRQSNGEAFQKYLEDTTKNLIKAMPAQQANLVLHA

SEQ ID NO: 46 - protein, 140 aa, Gossypium barbadense
MIPQQKKKKKQSYFKIASDSSAAQQMAKSTNYHPALSEFDKVKVLEESSPSKSKSKTIKELVTMSSKLDSLEKGESFLREKIQAQKLKYNDKPDSLRQSNGEAFQKYLEDTTKNLIKAMPAQQANLVLHAEQKLISEEDL

SEQ ID NO: 47 - protein, 140 aa, Gossypium barbadense
EQKLISEEDLMIPQQKKKKKQSYFKIASDSSAAQQMAKSTNYHPALSEFDKVKVLEESSPSKSKSKTIKELVTMSSKLDSLEKGESFLREKIQAQKLKYNDKPDSLRQSNGEAFQKYLEDTTKNLIKAMPAQQANLVLHA

SEQ ID NO: 48 - protein, 135 aa, Gossypium barbadense
QQMMIPKEAFFKSDSQSYIASPFSRMKASTPALLEFDYYHKVKVSALEEPSKSKSKTIKELVTMSSKLDSLEKGESFLREKIQAQKLKYNDKPDSLRQSNGEAFQKYLEDTTKNLIKAMPNLAKNLVLHARRRRR

SEQ ID NO: 49 - protein, 135 aa, Gossypium barbadense
RRRRRQQMMIPKEAFFKSDSQSYIASPFSRMKASTPALLEFDYYHKVKVSALEEPSKSKSKTIKELVTMSSKLDSLEKGESFLREKIQAQKLKYNDKPDSLRQSNGEAFQKYLEDTTKNLIKAMPNLAKNLVLHA

SEQ ID NO: 50 - protein, 136 aa, Gossypium barbadense
QQMMIPKEAFFKSDSQSYIASPFSRMKASTPALLEFDYYHKVKVSALEEPSKSKSKTIKELVTMSSKLDSLEKGESFLREKIQAQKLKYNDKPDSLRQSNGEAFQKYLEDTTKNLIKAMPNLAKNLVLHARRRRRR

SEQ ID NO: 51 - protein, 136 aa, Gossypium barbadense
RRRRRRQQMMIPKEAFFKSDSQSYIASPFSRMKASTPALLEFDYYHKVKVSALEEPSKSKSKTIKELVTMSSKLDSLEKGESFLREKIQAQKLKYNDKPDSLRQSNGEAFQKYLEDTTKNLIKAMPNLAKNLVLHA

SEQ ID NO: 52 - protein, 132 aa, Gossypium barbadense
QQMMIPKEAFFKSDSQSYIASPFSRMKASTPALLEFDYYHKVKVSALEEPSKSKSKTIKELVTMSSKLDSLEKGESFLREKIQAQKLKYNDKPDSLRQSNGEAFQKYLEDTTKNLIKAMPNLAKNLVLHAHH

SEQ ID NO: 53 - protein, 140 aa, Gossypium barbadense
HHHHHHHHHHQQMMIPKEAFFKSDSQSYIASPFSRMKASTPALLEFDYYHKVKVSALEEPSKSKSKTIKELVTMSSKLDSLEKGESFLREKIQAQKLKYNDKPDSLRQSNGEAFQKYLEDTTKNLIKAMPNLAKNLVLHA

SEQ ID NO: 54 - protein, 134 aa, Gossypium barbadense
QQMMIPKEAFFKSDSQSYIASPFSRMKASTPALLEFDYYHKVKVSALEEPSKSKSKTIKELVTMSSKLDSLEKGESFLREKIQAQKLKYNDKPDSLRQSNGEAFQKYLEDTTKNLIKAMPNLAKNLVLHAHHHH

SEQ ID NO: 55 - protein, 132 aa, Gossypium barbadense
HHQQMMIPKEAFFKSDSQSYIASPFSRMKASTPALLEFDYYHKVKVSALEEPSKSKSKTIKELVTMSSKLDSLEKGESFLREKIQAQKLKYNDKPDSLRQSNGEAFQKYLEDTTKNLIKAMPNLAKNLVLHA

SEQ ID NO: 56 - protein, 137 aa, Gossypium barbadense
HHHHHHHQQMMIPKEAFFKSDSQSYIASPFSRMKASTPALLEFDYYHKVKVSALEEPSKSKSKTIKELVTMSSKLDSLEKGESFLREKIQAQKLKYNDKPDSLRQSNGEAFQKYLEDTTKNLIKAMPNLAKNLVLHA

SEQ ID NO: 57 - protein, 140 aa, Gossypium barbadense
QQMMIPKEAFFKSDSQSYIASPFSRMKASTPALLEFDYYHKVKVSALEEPSKSKSKTIKELVTMSSKLDSLEKGESFLREKIQAQKLKYNDKPDSLRQSNGEAFQKYLEDTTKNLIKAMPNLAKNLVLHAHHHHHHHHHH

SEQ ID NO: 58 - protein, 138 aa, Gossypium barbadense
QQMMIPKEAFFKSDSQSYIASPFSRMKASTPALLEFDYYHKVKVSALEEPSKSKSKTIKELVTMSSKLDSLEKGESFLREKIQAQKLKYNDKPDSLRQSNGEAFQKYLEDTTKNLIKAMPNLAKNLVLHADYKDDDDK

SEQ ID NO: 59 - protein, 138 aa, Gossypium barbadense
DYKDDDDKQQMMIPKEAFFKSDSQSYIASPFSRMKASTPALLEFDYYHKVKVSALEEPSKSKSKTIKELVTMSSKLDSLEKGESFLREKIQAQKLKYNDKPDSLRQSNGEAFQKYLEDTTKNLIKAMPNLAKNLVLHA

SEQ ID NO: 60 - protein, 138 aa, Gossypium barbadense
QQMMIPKEAFFKSDSQSYIASPFSRMKASTPALLEFDYYHKVKVSALEEPSKSKSKTIKELVTMSSKLDSLEKGESFLREKIQAQKLKYNDKPDSLRQSNGEAFQKYLEDTTKNLIKAMPNLAKNLVLHAWSHPQFEK

SEQ ID NO: 61 - protein, 138 aa, Gossypium barbadense
WSHPQFEKQQMMIPKEAFFKSDSQSYIASPFSRMKASTPALLEFDYYHKVKVSALEEPSKSKSKTIKELVTMSSKLDSLEKGESFLREKIQAQKLKYNDKPDSLRQSNGEAFQKYLEDTTKNLIKAMPNLAKNLVLHA

SEQ ID NO: 62 - protein, 140 aa, Gossypium barbadense
QQMMIPKEAFFKSDSQSYIASPFSRMKASTPALLEFDYYHKVKVSALEEPSKSKSKTIKELVTMSSKLDSLEKGESFLREKIQAQKLKYNDKPDSLRQSNGEAFQKYLEDTTKNLIKAMPNLAKNLVLHAEQKLISEEDL

SEQ ID NO: 63 - protein, 140 aa, Gossypium barbadense
EQKLISEEDLQQMMIPKEAFFKSDSQSYIASPFSRMKASTPALLEFDYYHKVKVSALEEPSKSKSKTIKELVTMSSKLDSLEKGESFLREKIQAQKLKYNDKPDSLRQSNGEAFQKYLEDTTKNLIKAMPNLAKNLVLHA

SEQ ID NO: 64 - protein, 135 aa, Gossypium barbadense
MIPQQMVEAFQSYLAFKSDSSPFSSMAKSTPALSFEDNYHSSLEKAKVEPSKSKSKTIKELVTMSSKLDSLEKGESFLREKIQAQKLKYNDKPDSLRQSNGEAFQKYLEDTTKNLIKAMPNLKANLLVHARRRRR

SEQ ID NO: 65 - protein, 135 aa, Gossypium barbadense
RRRRRMIPQQMVEAFQSYLAFKSDSSPFSSMAKSTPALSFEDNYHSSLEKAKVEPSKSKSKTIKELVTMSSKLDSLEKGESFLREKIQAQKLKYNDKPDSLRQSNGEAFQKYLEDTTKNLIKAMPNLKANLLVHA

SEQ ID NO: 66 - protein, 136 aa, Gossypium barbadense
MIPQQMVEAFQSYLAFKSDSSPFSSMAKSTPALSFEDNYHSSLEKAKVEPSKSKSKTIKELVTMSSKLDSLEKGESFLREKIQAQKLKYNDKPDSLRQSNGEAFQKYLEDTTKNLIKAMPNLKANLLVHARRRRRR

SEQ ID NO: 67 - protein, 136 aa, Gossypium barbadense
RRRRRRMIPQQMVEAFQSYLAFKSDSSPFSSMAKSTPALSFEDNYHSSLEKAKVEPSKSKSKTIKELVTMSSKLDSLEKGESFLREKIQAQKLKYNDKPDSLRQSNGEAFQKYLEDTTKNLIKAMPNLKANLLVHA

SEQ ID NO: 68 - protein, 132 aa, Gossypium barbadense
MIPQQMVEAFQSYLAFKSDSSPFSSMAKSTPALSFEDNYHSSLEKAKVEPSKSKSKTIKELVTMSSKLDSLEKGESFLREKIQAQKLKYNDKPDSLRQSNGEAFQKYLEDTTKNLIKAMPNLKANLLVHAHH

SEQ ID NO: 69 - protein, 140 aa, Gossypium barbadense
HHHHHHHHHHMIPQQMVEAFQSYLAFKSDSSPFSSMAKSTPALSFEDNYHSSLEKAKVEPSKSKSKTIKELVTMSSKLDSLEKGESFLREKIQAQKLKYNDKPDSLRQSNGEAFQKYLEDTTKNLIKAMPNLKANLLVHA

SEQ ID NO: 70 - protein, 134 aa, Gossypium barbadense
MIPQQMVEAFQSYLAFKSDSSPFSSMAKSTPALSFEDNYHSSLEKAKVEPSKSKSKTIKELVTMSSKLDSLEKGESFLREKIQAQKLKYNDKPDSLRQSNGEAFQKYLEDTTKNLIKAMPNLKANLLVHAHHHH

SEQ ID NO: 71 - protein, 132 aa, Gossypium barbadense
HHMIPQQMVEAFQSYLAFKSDSSPFSSMAKSTPALSFEDNYHSSLEKAKVEPSKSKSKTIKELVTMSSKLDSLEKGESFLREKIQAQKLKYNDKPDSLRQSNGEAFQKYLEDTTKNLIKAMPNLKANLLVHA

SEQ ID NO: 72 - protein, 137 aa, Gossypium barbadense
HHHHHHHMIPQQMVEAFQSYLAFKSDSSPFSSMAKSTPALSFEDNYHSSLEKAKVEPSKSKSKTIKELVTMSSKLDSLEKGESFLREKIQAQKLKYNDKPDSLRQSNGEAFQKYLEDTTKNLIKAMPNLKANLLVHA

SEQ ID NO: 73 - protein, 140 aa, Gossypium barbadense
MIPQQMVEAFQSYLAFKSDSSPFSSMAKSTPALSFEDNYHSSLEKAKVEPSKSKSKTIKELVTMSSKLDSLEKGESFLREKIQAQKLKYNDKPDSLRQSNGEAFQKYLEDTTKNLIKAMPNLKANLLVHAHHHHHHHHHH

SEQ ID NO: 74 - protein, 138 aa, Gossypium barbadense
MIPQQMVEAFQSYLAFKSDSSPFSSMAKSTPALSFEDNYHSSLEKAKVEPSKSKSKTIKELVTMSSKLDSLEKGESFLREKIQAQKLKYNDKPDSLRQSNGEAFQKYLEDTTKNLIKAMPNLKANLLVHADYKDDDDK

SEQ ID NO: 75 - protein, 138 aa, Gossypium barbadense
DYKDDDDKMIPQQMVEAFQSYLAFKSDSSPFSSMAKSTPALSFEDNYHSSLEKAKVEPSKSKSKTIKELVTMSSKLDSLEKGESFLREKIQAQKLKYNDKPDSLRQSNGEAFQKYLEDTTKNLIKAMPNLKANLLVHA

SEQ ID NO: 76 - protein, 138 aa, Gossypium barbadense
MIPQQMVEAFQSYLAFKSDSSPFSSMAKSTPALSFEDNYHSSLEKAKVEPSKSKSKTIKELVTMSSKLDSLEKGESFLREKIQAQKLKYNDKPDSLRQSNGEAFQKYLEDTTKNLIKAMPNLKANLLVHAWSHPQFEK

SEQ ID NO: 77 - protein, 138 aa, Gossypium barbadense
WSHPQFEKMIPQQMVEAFQSYLAFKSDSSPFSSMAKSTPALSFEDNYHSSLEKAKVEPSKSKSKTIKELVTMSSKLDSLEKGESFLREKIQAQKLKYNDKPDSLRQSNGEAFQKYLEDTTKNLIKAMPNLKANLLVHA

SEQ ID NO: 78 - protein, 140 aa, Gossypium barbadense
MIPQQMVEAFQSYLAFKSDSSPFSSMAKSTPALSFEDNYHSSLEKAKVEPSKSKSKTIKELVTMSSKLDSLEKGESFLREKIQAQKLKYNDKPDSLRQSNGEAFQKYLEDTTKNLIKAMPNLKANLLVHAEQKLISEEDL

SEQ ID NO: 79 - protein, 140 aa, Gossypium barbadense
EQKLISEEDLMIPQQMVEAFQSYLAFKSDSSPFSSMAKSTPALSFEDNYHSSLEKAKVEPSKSKSKTIKELVTMSSKLDSLEKGESFLREKIQAQKLKYNDKPDSLRQSNGEAFQKYLEDTTKNLIKAMPNLKANLLVHA

SEQ ID NO: 80 - protein, 135 aa, Gossypium barbadense
MIPQQMKEAFQSYIAFKSDSMAKSTSPFSRPALSEFDNYHKAKVSSLFEPSKSKSKTIKELVTMSSKLDSLEKGESFLREKIQAQKLKYNDKPDSLRQSNGEAFQKYLEDTTKNLIKAMPNLKANLVLHARRRRR

SEQ ID NO: 81 - protein, 135 aa, Gossypium barbadense
RRRRRMIPQQMKEAFQSYIAFKSDSMAKSTSPFSRPALSEFDNYHKAKVSSLFEPSKSKSKTIKELVTMSSKLDSLEKGESFLREKIQAQKLKYNDKPDSLRQSNGEAFQKYLEDTTKNLIKAMPNLKANLVLHA

SEQ ID NO: 82 - protein, 136 aa, Gossypium barbadense
MIPQQMKEAFQSYIAFKSDSMAKSTSPFSRPALSEFDNYHKAKVSSLFEPSKSKSKTIKELVTMSSKLDSLEKGESFLREKIQAQKLKYNDKPDSLRQSNGEAFQKYLEDTTKNLIKAMPNLKANLVLHARRRRRR

SEQ ID NO: 83 - protein, 136 aa, Gossypium barbadense
RRRRRRMIPQQMKEAFQSYIAFKSDSMAKSTSPFSRPALSEFDNYHKAKVSSLFEPSKSKSKTIKELVTMSSKLDSLEKGESFLREKIQAQKLKYNDKPDSLRQSNGEAFQKYLEDTTKNLIKAMPNLKANLVLHA

SEQ ID NO: 84 - protein, 132 aa, Gossypium barbadense
MIPQQMKEAFQSYIAFKSDSMAKSTSPFSRPALSEFDNYHKAKVSSLFEPSKSKSKTIKELVTMSSKLDSLEKGESFLREKIQAQKLKYNDKPDSLRQSNGEAFQKYLEDTTKNLIKAMPNLKANLVLHAHH

SEQ ID NO: 85 - protein, 140 aa, Gossypium barbadense
HHHHHHHHHHMIPQQMKEAFQSYIAFKSDSMAKSTSPFSRPALSEFDNYHKAKVSSLFEPSKSKSKTIKELVTMSSKLDSLEKGESFLREKIQAQKLKYNDKPDSLRQSNGEAFQKYLEDTTKNLIKAMPNLKANLVLHA

SEQ ID NO: 86 - protein, 134 aa, Gossypium barbadense
MIPQQMKEAFQSYIAFKSDSMAKSTSPFSRPALSEFDNYHKAKVSSLFEPSKSKSKTIKELVTMSSKLDSLEKGESFLREKIQAQKLKYNDKPDSLRQSNGEAFQKYLEDTTKNLIKAMPNLKANLVLHAHHHH

SEQ ID NO: 87 - protein, 132 aa, Gossypium barbadense
HHMIPQQMKEAFQSYIAFKSDSMAKSTSPFSRPALSEFDNYHKAKVSSLFEPSKSKSKTIKELVTMSSKLDSLEKGESFLREKIQAQKLKYNDKPDSLRQSNGEAFQKYLEDTTKNLIKAMPNLKANLVLHA

SEQ ID NO: 88 - protein, 137 aa, Gossypium barbadense
HHHHHHHMIPQQMKEAFQSYIAFKSDSMAKSTSPFSRPALSEFDNYHKAKVSSLFEPSKSKSKTIKELVTMSSKLDSLEKGESFLREKIQAQKLKYNDKPDSLRQSNGEAFQKYLEDTTKNLIKAMPNLKANLVLHA

SEQ ID NO: 89 - protein, 140 aa, Gossypium barbadense
MIPQQMKEAFQSYIAFKSDSMAKSTSPFSRPALSEFDNYHKAKVSSLFEPSKSKSKTIKELVTMSSKLDSLEKGESFLREKIQAQKLKYNDKPDSLRQSNGEAFQKYLEDTTKNLIKAMPNLKANLVLHAHHHHHHHHHH

SEQ ID NO: 90 - protein, 138 aa, Gossypium barbadense
MIPQQMKEAFQSYIAFKSDSMAKSTSPFSRPALSEFDNYHKAKVSSLFEPSKSKSKTIKELVTMSSKLDSLEKGESFLREKIQAQKLKYNDKPDSLRQSNGEAFQKYLEDTTKNLIKAMPNLKANLVLHADYKDDDDK

SEQ ID NO: 91 - protein, 138 aa, Gossypium barbadense
DYKDDDDKMIPQQMKEAFQSYIAFKSDSMAKSTSPFSRPALSEFDNYHKAKVSSLFEPSKSKSKTIKELVTMSSKLDSLEKGESFLREKIQAQKLKYNDKPDSLRQSNGEAFQKYLEDTTKNLIKAMPNLKANLVLHA

SEQ ID NO: 92 - protein, 138 aa, Gossypium barbadense
MIPQQMKEAFQSYIAFKSDSMAKSTSPFSRPALSEFDNYHKAKVSSLFEPSKSKSKTIKELVTMSSKLDSLEKGESFLREKIQAQKLKYNDKPDSLRQSNGEAFQKYLEDTTKNLIKAMPNLKANLVLHAWSHPQFEK

SEQ ID NO: 93 - protein, 138 aa, Gossypium barbadense
WSHPQFEKMIPQQMKEAFQSYIAFKSDSMAKSTSPFSRPALSEFDNYHKAKVSSLFEPSKSKSKTIKELVTMSSKLDSLEKGESFLREKIQAQKLKYNDKPDSLRQSNGEAFQKYLEDTTKNLIKAMPNLKANLVLHA

SEQ ID NO: 94 - protein, 140 aa, Gossypium barbadense
MIPQQMKEAFQSYIAFKSDSMAKSTSPFSRPALSEFDNYHKAKVSSLFEPSKSKSKTIKELVTMSSKLDSLEKGESFLREKIQAQKLKYNDKPDSLRQSNGEAFQKYLEDTTKNLIKAMPNLKANLVLHAEQKLISEEDL

SEQ ID NO: 95 - protein, 140 aa, Gossypium barbadense
EQKLISEEDLMIPQQMKEAFQSYIAFKSDSMAKSTSPFSRPALSEFDNYHKAKVSSLFEPSKSKSKTIKELVTMSSKLDSLEKGESFLREKIQAQKLKYNDKPDSLRQSNGEAFQKYLEDTTKNLIKAMPNLKANLVLHA

SEQ ID NO: 96 - protein, 135 aa, Gossypium barbadense
MIPQPMKEAFQSYIAFKSDSSPFSVMAKSTPALSEFDNYHKAKVSALEEPSKSKSKTIKELVTMSSKLDSLEKGESFLREKIQAQKLKYNDKPDSLRQSNGEAFQKYLEDTTKNLIKAMPNLKAMLVLHARRRRR

SEQ ID NO: 97 - protein, 135 aa, Gossypium barbadense
RRRRRMIPQPMKEAFQSYIAFKSDSSPFSVMAKSTPALSEFDNYHKAKVSALEEPSKSKSKTIKELVTMSSKLDSLEKGESFLREKIQAQKLKYNDKPDSLRQSNGEAFQKYLEDTTKNLIKAMPNLKAMLVLHA

SEQ ID NO: 98 - protein, 136 aa, Gossypium barbadense
MIPQPMKEAFQSYIAFKSDSSPFSVMAKSTPALSEFDNYHKAKVSALEEPSKSKSKTIKELVTMSSKLDSLEKGESFLREKIQAQKLKYNDKPDSLRQSNGEAFQKYLEDTTKNLIKAMPNLKAMLVLHARRRRRR

SEQ ID NO: 99 - protein, 136 aa, Gossypium barbadense
RRRRRRMIPQPMKEAFQSYIAFKSDSSPFSVMAKSTPALSEFDNYHKAKVSALEEPSKSKSKTIKELVTMSSKLDSLEKGESFLREKIQAQKLKYNDKPDSLRQSNGEAFQKYLEDTTKNLIKAMPNLKAMLVLHA

SEQ ID NO: 100 - protein, 132 aa, Gossypium barbadense
MIPQPMKEAFQSYIAFKSDSSPFSVMAKSTPALSEFDNYHKAKVSALEEPSKSKSKTIKELVTMSSKLDSLEKGESFLREKIQAQKLKYNDKPDSLRQSNGEAFQKYLEDTTKNLIKAMPNLKAMLVLHAHH

SEQ ID NO: 101 - protein, 140 aa, Gossypium barbadense
HHHHHHHHHHMIPQPMKEAFQSYIAFKSDSSPFSVMAKSTPALSEFDNYHKAKVSALEEPSKSKSKTIKELVTMSSKLDSLEKGESFLREKIQAQKLKYNDKPDSLRQSNGEAFQKYLEDTTKNLIKAMPNLKAMLVLHA

SEQ ID NO: 102 - protein, 134 aa, Gossypium barbadense
MIPQPMKEAFQSYIAFKSDSSPFSVMAKSTPALSEFDNYHKAKVSALEEPSKSKSKTIKELVTMSSKLDSLEKGESFLREKIQAQKLKYNDKPDSLRQSNGEAFQKYLEDTTKNLIKAMPNLKAMLVLHAHHHH

SEQ ID NO: 103 - protein, 132 aa, Gossypium barbadense
HHMIPQPMKEAFQSYIAFKSDSSPFSVMAKSTPALSEFDNYHKAKVSALEEPSKSKSKTIKELVTMSSKLDSLEKGESFLREKIQAQKLKYNDKPDSLRQSNGEAFQKYLEDTTKNLIKAMPNLKAMLVLHA

SEQ ID NO: 104 - protein, 137 aa, Gossypium barbadense
HHHHHHHMIPQPMKEAFQSYIAFKSDSSPFSVMAKSTPALSEFDNYHKAKVSALEEPSKSKSKTIKELVTMSSKLDSLEKGESFLREKIQAQKLKYNDKPDSLRQSNGEAFQKYLEDTTKNLIKAMPNLKAMLVLHA

SEQ ID NO: 105 - protein, 140 aa, Gossypium barbadense
MIPQPMKEAFQSYIAFKSDSSPFSVMAKSTPALSEFDNYHKAKVSALEEPSKSKSKTIKELVTMSSKLDSLEKGESFLREKIQAQKLKYNDKPDSLRQSNGEAFQKYLEDTTKNLIKAMPNLKAMLVLHAHHHHHHHHHH

SEQ ID NO: 106 - protein, 138 aa, Gossypium barbadense
MIPQPMKEAFQSYIAFKSDSSPFSVMAKSTPALSEFDNYHKAKVSALEEPSKSKSKTIKELVTMSSKLDSLEKGESFLREKIQAQKLKYNDKPDSLRQSNGEAFQKYLEDTTKNLIKAMPNLKAMLVLHADYKDDDDK

SEQ ID NO: 107 - protein, 138 aa, Gossypium barbadense
DYKDDDDKMIPQPMKEAFQSYIAFKSDSSPFSVMAKSTPALSEFDNYHKAKVSALEEPSKSKSKTIKELVTMSSKLDSLEKGESFLREKIQAQKLKYNDKPDSLRQSNGEAFQKYLEDTTKNLIKAMPNLKAMLVLHA

SEQ ID NO: 108 - protein, 138 aa, Gossypium barbadense
MIPQPMKEAFQSYIAFKSDSSPFSVMAKSTPALSEFDNYHKAKVSALEEPSKSKSKTIKELVTMSSKLDSLEKGESFLREKIQAQKLKYNDKPDSLRQSNGEAFQKYLEDTTKNLIKAMPNLKAMLVLHAWSHPQFEK

SEQ ID NO: 109 - protein, 138 aa, Gossypium barbadense
WSHPQFEKMIPQPMKEAFQSYIAFKSDSSPFSVMAKSTPALSEFDNYHKAKVSALEEPSKSKSKTIKELVTMSSKLDSLEKGESFLREKIQAQKLKYNDKPDSLRQSNGEAFQKYLEDTTKNLIKAMPNLKAMLVLHA

SEQ ID NO: 110 - protein, 140 aa, Gossypium barbadense
MIPQPMKEAFQSYIAFKSDSSPFSVMAKSTPALSEFDNYHKAKVSALEEPSKSKSKTIKELVTMSSKLDSLEKGESFLREKIQAQKLKYNDKPDSLRQSNGEAFQKYLEDTTKNLIKAMPNLKAMLVLHAEQKLISEEDL

SEQ ID NO: 111 - protein, 140 aa, Gossypium barbadense
EQKLISEEDLMIPQPMKEAFQSYIAFKSDSSPFSVMAKSTPALSEFDNYHKAKVSALEEPSKSKSKTIKELVTMSSKLDSLEKGESFLREKIQAQKLKYNDKPDSLRQSNGEAFQKYLEDTTKNLIKAMPNLKAMLVLHA

SEQ ID NO: 112 - protein, 135 aa, Gossypium barbadense
MPPQAMKLFFQSVIAKKSLSSPVSSSATSTPAISGFDNMIKAKASSLEEPSKEKSKTIKQIVTMSSKLMSLEKGESQLRVKLRMQKLKYNKKKDSLRQSNPEAFQKYLEDTTKNVIKMQVNRKANLVLHARRRRR

SEQ ID NO: 113 - protein, 135 aa, Gossypium barbadense
RRRRRMPPQAMKLFFQSVIAKKSLSSPVSSSATSTPAISGFDNMIKAKASSLEEPSKEKSKTIKQIVTMSSKLMSLEKGESQLRVKLRMQKLKYNKKKDSLRQSNPEAFQKYLEDTTKNVIKMQVNRKANLVLHA

SEQ ID NO: 114 - protein, 136 aa, Gossypium barbadense
MPPQAMKLFFQSVIAKKSLSSPVSSSATSTPAISGFDNMIKAKASSLEEPSKEKSKTIKQIVTMSSKLMSLEKGESQLRVKLRMQKLKYNKKKDSLRQSNPEAFQKYLEDTTKNVIKMQVNRKANLVLHARRRRRR

SEQ ID NO: 115 - protein, 136 aa, Gossypium barbadense
RRRRRRMPPQAMKLFFQSVIAKKSLSSPVSSSATSTPAISGFDNMIKAKASSLEEPSKEKSKTIKQIVTMSSKLMSLEKGESQLRVKLRMQKLKYNKKKDSLRQSNPEAFQKYLEDTTKNVIKMQVNRKANLVLHA

SEQ ID NO: 116 - protein, 132 aa, Gossypium barbadense
MPPQAMKLFFQSVIAKKSLSSPVSSSATSTPAISGFDNMIKAKASSLEEPSKEKSKTIKQIVTMSSKLMSLEKGESQLRVKLRMQKLKYNKKKDSLRQSNPEAFQKYLEDTTKNVIKMQVNRKANLVLHAHH

SEQ ID NO: 117 - protein, 140 aa, Gossypium barbadense
HHHHHHHHHHMPPQAMKLFFQSVIAKKSLSSPVSSSATSTPAISGFDNMIKAKASSLEEPSKEKSKTIKQIVTMSSKLMSLEKGESQLRVKLRMQKLKYNKKKDSLRQSNPEAFQKYLEDTTKNVIKMQVNRKANLVLHA

SEQ ID NO: 118 - protein, 134 aa, Gossypium barbadense
MPPQAMKLFFQSVIAKKSLSSPVSSSATSTPAISGFDNMIKAKASSLEEPSKEKSKTIKQIVTMSSKLMSLEKGESQLRVKLRMQKLKYNKKKDSLRQSNPEAFQKYLEDTTKNVIKMQVNRKANLVLHAHHHH

SEQ ID NO: 119 - protein, 132 aa, Gossypium barbadense
HHMPPQAMKLFFQSVIAKKSLSSPVSSSATSTPAISGFDNMIKAKASSLEEPSKEKSKTIKQIVTMSSKLMSLEKGESQLRVKLRMQKLKYNKKKDSLRQSNPEAFQKYLEDTTKNVIKMQVNRKANLVLHA

SEQ ID NO: 120 - protein, 137 aa, Gossypium barbadense
HHHHHHHMPPQAMKLFFQSVIAKKSLSSPVSSSATSTPAISGFDNMIKAKASSLEEPSKEKSKTIKQIVTMSSKLMSLEKGESQLRVKLRMQKLKYNKKKDSLRQSNPEAFQKYLEDTTKNVIKMQVNRKANLVLHA

SEQ ID NO: 121 - protein, 140 aa, Gossypium barbadense
MPPQAMKLFFQSVIAKKSLSSPVSSSATSTPAISGFDNMIKAKASSLEEPSKEKSKTIKQIVTMSSKLMSLEKGESQLRVKLRMQKLKYNKKKDSLRQSNPEAFQKYLEDTTKNVIKMQVNRKANLVLHAHHHHHHHHHH

SEQ ID NO: 122 - protein, 138 aa, Gossypium barbadense
MPPQAMKLFFQSVIAKKSLSSPVSSSATSTPAISGFDNMIKAKASSLEEPSKEKSKTIKQIVTMSSKLMSLEKGESQLRVKLRMQKLKYNKKKDSLRQSNPEAFQKYLEDTTKNVIKMQVNRKANLVLHADYKDDDDK

SEQ ID NO: 123 - protein, 138 aa, Gossypium barbadense
DYKDDDDKMPPQAMKLFFQSVIAKKSLSSPVSSSATSTPAISGFDNMIKAKASSLEEPSKEKSKTIKQIVTMSSKLMSLEKGESQLRVKLRMQKLKYNKKKDSLRQSNPEAFQKYLEDTTKNVIKMQVNRKANLVLHA

SEQ ID NO: 124 - protein, 138 aa, Gossypium barbadense
MPPQAMKLFFQSVIAKKSLSSPVSSSATSTPAISGFDNMIKAKASSLEEPSKEKSKTIKQIVTMSSKLMSLEKGESQLRVKLRMQKLKYNKKKDSLRQSNPEAFQKYLEDTTKNVIKMQVNRKANLVLHAWSHPQFEK

SEQ ID NO: 125 - protein, 138 aa, Gossypium barbadense
WSHPQFEKMPPQAMKLFFQSVIAKKSLSSPVSSSATSTPAISGFDNMIKAKASSLEEPSKEKSKTIKQIVTMSSKLMSLEKGESQLRVKLRMQKLKYNKKKDSLRQSNPEAFQKYLEDTTKNVIKMQVNRKANLVLHA

SEQ ID NO: 126 - protein, 140 aa, Gossypium barbadense
MPPQAMKLFFQSVIAKKSLSSPVSSSATSTPAISGFDNMIKAKASSLEEPSKEKSKTIKQIVTMSSKLMSLEKGESQLRVKLRMQKLKYNKKKDSLRQSNPEAFQKYLEDTTKNVIKMQVNRKANLVLHAEQKLISEEDL

SEQ ID NO: 127 - protein, 140 aa, Gossypium barbadense
EQKLISEEDLMPPQAMKLFFQSVIAKKSLSSPVSSSATSTPAISGFDNMIKAKASSLEEPSKEKSKTIKQIVTMSSKLMSLEKGESQLRVKLRMQKLKYNKKKDSLRQSNPEAFQKYLEDTTKNVIKMQVNRKANLVLHA

SEQ ID NO: 128 - protein, 135 aa, Gossypium barbadense
MPPQQMKLFFQSVIAFKSLSSPVSRMATSTPAISGFDNMIKAKASSLEEPSKEKSKTIKQIVTMSSKLMSLEKGESFLRVKLRMQKLKYNDKPDSLRQSNGEAFQKYLEDTTKNVIKMQVNRKANLVLHARRRRR

SEQ ID NO: 129 - protein, 135 aa, Gossypium barbadense
RRRRRMPPQQMKLFFQSVIAFKSLSSPVSRMATSTPAISGFDNMIKAKASSLEEPSKEKSKTIKQIVTMSSKLMSLEKGESFLRVKLRMQKLKYNDKPDSLRQSNGEAFQKYLEDTTKNVIKMQVNRKANLVLHA

SEQ ID NO: 130 - protein, 136 aa, Gossypium barbadense
MPPQQMKLFFQSVIAFKSLSSPVSRMATSTPAISGFDNMIKAKASSLEEPSKEKSKTIKQIVTMSSKLMSLEKGESFLRVKLRMQKLKYNDKPDSLRQSNGEAFQKYLEDTTKNVIKMQVNRKANLVLHARRRRRR

SEQ ID NO: 131 - protein, 136 aa, Gossypium barbadense
RRRRRRMPPQQMKLFFQSVIAFKSLSSPVSRMATSTPAISGFDNMIKAKASSLEEPSKEKSKTIKQIVTMSSKLMSLEKGESFLRVKLRMQKLKYNDKPDSLRQSNGEAFQKYLEDTTKNVIKMQVNRKANLVLHA

SEQ ID NO: 132 - protein, 132 aa, Gossypium barbadense
MPPQQMKLFFQSVIAFKSLSSPVSRMATSTPAISGFDNMIKAKASSLEEPSKEKSKTIKQIVTMSSKLMSLEKGESFLRVKLRMQKLKYNDKPDSLRQSNGEAFQKYLEDTTKNVIKMQVNRKANLVLHAHH

SEQ ID NO: 133 - protein, 140 aa, Gossypium barbadense
HHHHHHHHHHMPPQQMKLFFQSVIAFKSLSSPVSRMATSTPAISGFDNMIKAKASSLEEPSKEKSKTIKQIVTMSSKLMSLEKGESFLRVKLRMQKLKYNDKPDSLRQSNGEAFQKYLEDTTKNVIKMQVNRKANLVLHA

SEQ ID NO: 134 - protein, 134 aa, Gossypium barbadense
MPPQQMKLFFQSVIAFKSLSSPVSRMATSTPAISGFDNMIKAKASSLEEPSKEKSKTIKQIVTMSSKLMSLEKGESFLRVKLRMQKLKYNDKPDSLRQSNGEAFQKYLEDTTKNVIKMQVNRKANLVLHAHHHH

SEQ ID NO: 135 - protein, 132 aa, Gossypium barbadense
HHMPPQQMKLFFQSVIAFKSLSSPVSRMATSTPAISGFDNMIKAKASSLEEPSKEKSKTIKQIVTMSSKLMSLEKGESFLRVKLRMQKLKYNDKPDSLRQSNGEAFQKYLEDTTKNVIKMQVNRKANLVLHA

SEQ ID NO: 136 - protein, 137 aa, Gossypium barbadense
HHHHHHHMPPQQMKLFFQSVIAFKSLSSPVSRMATSTPAISGFDNMIKAKASSLEEPSKEKSKTIKQIVTMSSKLMSLEKGESFLRVKLRMQKLKYNDKPDSLRQSNGEAFQKYLEDTTKNVIKMQVNRKANLVLHA

SEQ ID NO: 137 - protein, 140 aa, Gossypium barbadense
MPPQQMKLFFQSVIAFKSLSSPVSRMATSTPAISGFDNMIKAKASSLEEPSKEKSKTIKQIVTMSSKLMSLEKGESFLRVKLRMQKLKYNDKPDSLRQSNGEAFQKYLEDTTKNVIKMQVNRKANLVLHAHHHHHHHHHH

SEQ ID NO: 138 - protein, 138 aa, Gossypium barbadense
MPPQQMKLFFQSVIAFKSLSSPVSRMATSTPAISGFDNMIKAKASSLEEPSKEKSKTIKQIVTMSSKLMSLEKGESFLRVKLRMQKLKYNDKPDSLRQSNGEAFQKYLEDTTKNVIKMQVNRKANLVLHADYKDDDDK

SEQ ID NO: 139 - protein, 138 aa, Gossypium barbadense
DYKDDDDKMPPQQMKLFFQSVIAFKSLSSPVSRMATSTPAISGFDNMIKAKASSLEEPSKEKSKTIKQIVTMSSKLMSLEKGESFLRVKLRMQKLKYNDKPDSLRQSNGEAFQKYLEDTTKNVIKMQVNRKANLVLHA

SEQ ID NO: 140 - protein, 138 aa, Gossypium barbadense
MPPQQMKLFFQSVIAFKSLSSPVSRMATSTPAISGFDNMIKAKASSLEEPSKEKSKTIKQIVTMSSKLMSLEKGESFLRVKLRMQKLKYNDKPDSLRQSNGEAFQKYLEDTTKNVIKMQVNRKANLVLHAWSHPQFEK

SEQ ID NO: 141 - protein, 138 aa, Gossypium barbadense
WSHPQFEKMPPQQMKLFFQSVIAFKSLSSPVSRMATSTPAISGFDNMIKAKASSLEEPSKEKSKTIKQIVTMSSKLMSLEKGESFLRVKLRMQKLKYNDKPDSLRQSNGEAFQKYLEDTTKNVIKMQVNRKANLVLHA

SEQ ID NO: 142 - protein, 140 aa, Gossypium barbadense
MPPQQMKLFFQSVIAFKSLSSPVSRMATSTPAISGFDNMIKAKASSLEEPSKEKSKTIKQIVTMSSKLMSLEKGESFLRVKLRMQKLKYNDKPDSLRQSNGEAFQKYLEDTTKNVIKMQVNRKANLVLHAEQKLISEEDL

SEQ ID NO: 143 - protein, 140 aa, Gossypium barbadense
EQKLISEEDLMPPQQMKLFFQSVIAFKSLSSPVSRMATSTPAISGFDNMIKAKASSLEEPSKEKSKTIKQIVTMSSKLMSLEKGESFLRVKLRMQKLKYNDKPDSLRQSNGEAFQKYLEDTTKNVIKMQVNRKANLVLHA

SEQ ID NO: 144 - protein, 135 aa, Gossypium barbadense
MIPQLMKGMFQSYIMFTSDDSPFSRMAVSTPALVEFDNYKKAKVSSLVSPSKSKSKTIKEVVTRSSKLDSLEKGESLLREKRQSQKLKYNDKPDSLRQSNGEAFQKYLEDTTKNLMKAMRVLKANLVLHARRRRR

SEQ ID NO: 145 - protein, 135 aa, Gossypium barbadense
RRRRRMIPQLMKGMFQSYIMFTSDDSPFSRMAVSTPALVEFDNYKKAKVSSLVSPSKSKSKTIKEVVTRSSKLDSLEKGESLLREKRQSQKLKYNDKPDSLRQSNGEAFQKYLEDTTKNLMKAMRVLKANLVLHA

SEQ ID NO: 146 - protein, 136 aa, Gossypium barbadense
MIPQLMKGMFQSYIMFTSDDSPFSRMAVSTPALVEFDNYKKAKVSSLVSPSKSKSKTIKEVVTRSSKLDSLEKGESLLREKRQSQKLKYNDKPDSLRQSNGEAFQKYLEDTTKNLMKAMRVLKANLVLHARRRRRR

SEQ ID NO: 147 - protein, 136 aa, Gossypium barbadense
RRRRRRMIPQLMKGMFQSYIMFTSDDSPFSRMAVSTPALVEFDNYKKAKVSSLVSPSKSKSKTIKEVVTRSSKLDSLEKGESLLREKRQSQKLKYNDKPDSLRQSNGEAFQKYLEDTTKNLMKAMRVLKANLVLHA

SEQ ID NO: 148 - protein, 132 aa, Gossypium barbadense
MIPQLMKGMFQSYIMFTSDDSPFSRMAVSTPALVEFDNYKKAKVSSLVSPSKSKSKTIKEVVTRSSKLDSLEKGESLLREKRQSQKLKYNDKPDSLRQSNGEAFQKYLEDTTKNLMKAMRVLKANLVLHAHH

SEQ ID NO: 149 - protein, 140 aa, Gossypium barbadense
HHHHHHHHHHMIPQLMKGMFQSYIMFTSDDSPFSRMAVSTPALVEFDNYKKAKVSSLVSPSKSKSKTIKEVVTRSSKLDSLEKGESLLREKRQSQKLKYNDKPDSLRQSNGEAFQKYLEDTTKNLMKAMRVLKANLVLHA

SEQ ID NO: 150 - protein, 134 aa, Gossypium barbadense
MIPQLMKGMFQSYIMFTSDDSPFSRMAVSTPALVEFDNYKKAKVSSLVSPSKSKSKTIKEVVTRSSKLDSLEKGESLLREKRQSQKLKYNDKPDSLRQSNGEAFQKYLEDTTKNLMKAMRVLKANLVLHAHHHH

SEQ ID NO: 151 - protein, 132 aa, Gossypium barbadense
HHMIPQLMKGMFQSYIMFTSDDSPFSRMAVSTPALVEFDNYKKAKVSSLVSPSKSKSKTIKEVVTRSSKLDSLEKGESLLREKRQSQKLKYNDKPDSLRQSNGEAFQKYLEDTTKNLMKAMRVLKANLVLHA

SEQ ID NO: 152 - protein, 137 aa, Gossypium barbadense
HHHHHHHMIPQLMKGMFQSYIMFTSDDSPFSRMAVSTPALVEFDNYKKAKVSSLVSPSKSKSKTIKEVVTRSSKLDSLEKGESLLREKRQSQKLKYNDKPDSLRQSNGEAFQKYLEDTTKNLMKAMRVLKANLVLHA

SEQ ID NO: 153 - protein, 140 aa, Gossypium barbadense
MIPQLMKGMFQSYIMFTSDDSPFSRMAVSTPALVEFDNYKKAKVSSLVSPSKSKSKTIKEVVTRSSKLDSLEKGESLLREKRQSQKLKYNDKPDSLRQSNGEAFQKYLEDTTKNLMKAMRVLKANLVLHAHHHHHHHHHH

SEQ ID NO: 154 - protein, 138 aa, Gossypium barbadense
MIPQLMKGMFQSYIMFTSDDSPFSRMAVSTPALVEFDNYKKAKVSSLVSPSKSKSKTIKEVVTRSSKLDSLEKGESLLREKRQSQKLKYNDKPDSLRQSNGEAFQKYLEDTTKNLMKAMRVLKANLVLHADYKDDDDK

SEQ ID NO: 155 - protein, 138 aa, Gossypium barbadense
DYKDDDDKMIPQLMKGMFQSYIMFTSDDSPFSRMAVSTPALVEFDNYKKAKVSSLVSPSKSKSKTIKEVVTRSSKLDSLEKGESLLREKRQSQKLKYNDKPDSLRQSNGEAFQKYLEDTTKNLMKAMRVLKANLVLHA

SEQ ID NO: 156 - protein, 138 aa, Gossypium barbadense
MIPQLMKGMFQSYIMFTSDDSPFSRMAVSTPALVEFDNYKKAKVSSLVSPSKSKSKTIKEVVTRSSKLDSLEKGESLLREKRQSQKLKYNDKPDSLRQSNGEAFQKYLEDTTKNLMKAMRVLKANLVLHAWSHPQFEK

SEQ ID NO: 157 - protein, 138 aa, Gossypium barbadense
WSHPQFEKMIPQLMKGMFQSYIMFTSDDSPFSRMAVSTPALVEFDNYKKAKVSSLVSPSKSKSKTIKEVVTRSSKLDSLEKGESLLREKRQSQKLKYNDKPDSLRQSNGEAFQKYLEDTTKNLMKAMRVLKANLVLHA

SEQ ID NO: 158 - protein, 140 aa, Gossypium barbadense
MIPQLMKGMFQSYIMFTSDDSPFSRMAVSTPALVEFDNYKKAKVSSLVSPSKSKSKTIKEVVTRSSKLDSLEKGESLLREKRQSQKLKYNDKPDSLRQSNGEAFQKYLEDTTKNLMKAMRVLKANLVLHAEQKLISEEDL

SEQ ID NO: 159 - protein, 140 aa, Gossypium barbadense
EQKLISEEDLMIPQLMKGMFQSYIMFTSDDSPFSRMAVSTPALVEFDNYKKAKVSSLVSPSKSKSKTIKEVVTRSSKLDSLEKGESLLREKRQSQKLKYNDKPDSLRQSNGEAFQKYLEDTTKNLMKAMRVLKANLVLHA

SEQ ID NO: 160 - protein, 135 aa, Gossypium barbadense
MIPQLMKKMFQSYIMFKSDSSPFSRMAVSTPALVEFDNYKKAKVSSLESPSKSKSKTIKEVVTRSSKLDSLEKGESFLREKRQSQKLKYNDKPDSLRQSNGEAFQKYLEDTTKNLMKAMRVLKANLVLHARRRRR

SEQ ID NO: 161 - protein, 135 aa, Gossypium barbadense
RRRRRMIPQLMKKMFQSYIMFKSDSSPFSRMAVSTPALVEFDNYKKAKVSSLESPSKSKSKTIKEVVTRSSKLDSLEKGESFLREKRQSQKLKYNDKPDSLRQSNGEAFQKYLEDTTKNLMKAMRVLKANLVLHA

SEQ ID NO: 162 - protein, 136 aa, Gossypium barbadense
MIPQLMKKMFQSYIMFKSDSSPFSRMAVSTPALVEFDNYKKAKVSSLESPSKSKSKTIKEVVTRSSKLDSLEKGESFLREKRQSQKLKYNDKPDSLRQSNGEAFQKYLEDTTKNLMKAMRVLKANLVLHARRRRRR

SEQ ID NO: 163 - protein, 136 aa, Gossypium barbadense
RRRRRRMIPQLMKKMFQSYIMFKSDSSPFSRMAVSTPALVEFDNYKKAKVSSLESPSKSKSKTIKEVVTRSSKLDSLEKGESFLREKRQSQKLKYNDKPDSLRQSNGEAFQKYLEDTTKNLMKAMRVLKANLVLHA

SEQ ID NO: 164 - protein, 132 aa, Gossypium barbadense
MIPQLMKKMFQSYIMFKSDSSPFSRMAVSTPALVEFDNYKKAKVSSLESPSKSKSKTIKEVVTRSSKLDSLEKGESFLREKRQSQKLKYNDKPDSLRQSNGEAFQKYLEDTTKNLMKAMRVLKANLVLHAHH

SEQ ID NO: 165 - protein, 140 aa, Gossypium barbadense
HHHHHHHHHHMIPQLMKKMFQSYIMFKSDSSPFSRMAVSTPALVEFDNYKKAKVSSLESPSKSKSKTIKEVVTRSSKLDSLEKGESFLREKRQSQKLKYNDKPDSLRQSNGEAFQKYLEDTTKNLMKAMRVLKANLVLHA

SEQ ID NO: 166 - protein, 134 aa, Gossypium barbadense
MIPQLMKKMFQSYIMFKSDSSPFSRMAVSTPALVEFDNYKKAKVSSLESPSKSKSKTIKEVVTRSSKLDSLEKGESFLREKRQSQKLKYNDKPDSLRQSNGEAFQKYLEDTTKNLMKAMRVLKANLVLHAHHHH

SEQ ID NO: 167 - protein, 132 aa, Gossypium barbadense
HHMIPQLMKKMFQSYIMFKSDSSPFSRMAVSTPALVEFDNYKKAKVSSLESPSKSKSKTIKEVVTRSSKLDSLEKGESFLREKRQSQKLKYNDKPDSLRQSNGEAFQKYLEDTTKNLMKAMRVLKANLVLHA

SEQ ID NO: 168 - protein, 137 aa, Gossypium barbadense
HHHHHHHMIPQLMKKMFQSYIMFKSDSSPFSRMAVSTPALVEFDNYKKAKVSSLESPSKSKSKTIKEVVTRSSKLDSLEKGESFLREKRQSQKLKYNDKPDSLRQSNGEAFQKYLEDTTKNLMKAMRVLKANLVLHA

SEQ ID NO: 169 - protein, 140 aa, Gossypium barbadense
MIPQLMKKMFQSYIMFKSDSSPFSRMAVSTPALVEFDNYKKAKVSSLESPSKSKSKTIKEVVTRSSKLDSLEKGESFLREKRQSQKLKYNDKPDSLRQSNGEAFQKYLEDTTKNLMKAMRVLKANLVLHAHHHHHHHHHH

SEQ ID NO: 170 - protein, 138 aa, Gossypium barbadense
MIPQLMKKMFQSYIMFKSDSSPFSRMAVSTPALVEFDNYKKAKVSSLESPSKSKSKTIKEVVTRSSKLDSLEKGESFLREKRQSQKLKYNDKPDSLRQSNGEAFQKYLEDTTKNLMKAMRVLKANLVLHADYKDDDDK

SEQ ID NO: 171 - protein, 138 aa, Gossypium barbadense
DYKDDDDKMIPQLMKKMFQSYIMFKSDSSPFSRMAVSTPALVEFDNYKKAKVSSLESPSKSKSKTIKEVVTRSSKLDSLEKGESFLREKRQSQKLKYNDKPDSLRQSNGEAFQKYLEDTTKNLMKAMRVLKANLVLHA

SEQ ID NO: 172 - protein, 138 aa, Gossypium barbadense
MIPQLMKKMFQSYIMFKSDSSPFSRMAVSTPALVEFDNYKKAKVSSLESPSKSKSKTIKEVVTRSSKLDSLEKGESFLREKRQSQKLKYNDKPDSLRQSNGEAFQKYLEDTTKNLMKAMRVLKANLVLHAWSHPQFEK

SEQ ID NO: 173 - protein, 138 aa, Gossypium barbadense
WSHPQFEKMIPQLMKKMFQSYIMFKSDSSPFSRMAVSTPALVEFDNYKKAKVSSLESPSKSKSKTIKEVVTRSSKLDSLEKGESFLREKRQSQKLKYNDKPDSLRQSNGEAFQKYLEDTTKNLMKAMRVLKANLVLHA

SEQ ID NO: 174 - protein, 140 aa, Gossypium barbadense
MIPQLMKKMFQSYIMFKSDSSPFSRMAVSTPALVEFDNYKKAKVSSLESPSKSKSKTIKEVVTRSSKLDSLEKGESFLREKRQSQKLKYNDKPDSLRQSNGEAFQKYLEDTTKNLMKAMRVLKANLVLHAEQKLISEEDL

SEQ ID NO: 175 - protein, 140 aa, Gossypium barbadense
EQKLISEEDLMIPQLMKKMFQSYIMFKSDSSPFSRMAVSTPALVEFDNYKKAKVSSLESPSKSKSKTIKEVVTRSSKLDSLEKGESFLREKRQSQKLKYNDKPDSLRQSNGEAFQKYLEDTTKNLMKAMRVLKANLVLHA

SEQ ID NO: 176 - protein, 135 aa, Gossypium barbadense
MIPQQMKLAFQSYIAFKSDSSPFSRMATSTPALSEFDNYHKAKVSSLEEPSKEKSKTIKELVTMSSKLDSLEKGESFLREKIRAQKLKYNDKPDSLRQSNGEAFQKYLEDTTKNLIKAQPNLKANLVLHARRRRR

SEQ ID NO: 177 - protein, 135 aa, Gossypium barbadense
RRRRRMIPQQMKLAFQSYIAFKSDSSPFSRMATSTPALSEFDNYHKAKVSSLEEPSKEKSKTIKELVTMSSKLDSLEKGESFLREKIRAQKLKYNDKPDSLRQSNGEAFQKYLEDTTKNLIKAQPNLKANLVLHA

SEQ ID NO: 178 - protein, 136 aa, Gossypium barbadense
MIPQQMKLAFQSYIAFKSDSSPFSRMATSTPALSEFDNYHKAKVSSLEEPSKEKSKTIKELVTMSSKLDSLEKGESFLREKIRAQKLKYNDKPDSLRQSNGEAFQKYLEDTTKNLIKAQPNLKANLVLHARRRRRR

SEQ ID NO: 179 - protein, 136 aa, Gossypium barbadense
RRRRRRMIPQQMKLAFQSYIAFKSDSSPFSRMATSTPALSEFDNYHKAKVSSLEEPSKEKSKTIKELVTMSSKLDSLEKGESFLREKIRAQKLKYNDKPDSLRQSNGEAFQKYLEDTTKNLIKAQPNLKANLVLHA

SEQ ID NO: 180 - protein, 132 aa, Gossypium barbadense
MIPQQMKLAFQSYIAFKSDSSPFSRMATSTPALSEFDNYHKAKVSSLEEPSKEKSKTIKELVTMSSKLDSLEKGESFLREKIRAQKLKYNDKPDSLRQSNGEAFQKYLEDTTKNLIKAQPNLKANLVLHAHH

SEQ ID NO: 181 - protein, 140 aa, Gossypium barbadense
HHHHHHHHHHMIPQQMKLAFQSYIAFKSDSSPFSRMATSTPALSEFDNYHKAKVSSLEEPSKEKSKTIKELVTMSSKLDSLEKGESFLREKIRAQKLKYNDKPDSLRQSNGEAFQKYLEDTTKNLIKAQPNLKANLVLHA

SEQ ID NO: 182 - protein, 134 aa, Gossypium barbadense
MIPQQMKLAFQSYIAFKSDSSPFSRMATSTPALSEFDNYHKAKVSSLEEPSKEKSKTIKELVTMSSKLDSLEKGESFLREKIRAQKLKYNDKPDSLRQSNGEAFQKYLEDTTKNLIKAQPNLKANLVLHAHHHH

SEQ ID NO: 183 - protein, 132 aa, Gossypium barbadense
HHMIPQQMKLAFQSYIAFKSDSSPFSRMATSTPALSEFDNYHKAKVSSLEEPSKEKSKTIKELVTMSSKLDSLEKGESFLREKIRAQKLKYNDKPDSLRQSNGEAFQKYLEDTTKNLIKAQPNLKANLVLHA

SEQ ID NO: 184 - protein, 137 aa, Gossypium barbadense
HHHHHHHMIPQQMKLAFQSYIAFKSDSSPFSRMATSTPALSEFDNYHKAKVSSLEEPSKEKSKTIKELVTMSSKLDSLEKGESFLREKIRAQKLKYNDKPDSLRQSNGEAFQKYLEDTTKNLIKAQPNLKANLVLHA

SEQ ID NO: 185 - protein, 140 aa, Gossypium barbadense
MIPQQMKLAFQSYIAFKSDSSPFSRMATSTPALSEFDNYHKAKVSSLEEPSKEKSKTIKELVTMSSKLDSLEKGESFLREKIRAQKLKYNDKPDSLRQSNGEAFQKYLEDTTKNLIKAQPNLKANLVLHAHHHHHHHHHH

SEQ ID NO: 186 - protein, 138 aa, Gossypium barbadense
MIPQQMKLAFQSYIAFKSDSSPFSRMATSTPALSEFDNYHKAKVSSLEEPSKEKSKTIKELVTMSSKLDSLEKGESFLREKIRAQKLKYNDKPDSLRQSNGEAFQKYLEDTTKNLIKAQPNLKANLVLHADYKDDDDK

SEQ ID NO: 187 - protein, 138 aa, Gossypium barbadense
DYKDDDDKMIPQQMKLAFQSYIAFKSDSSPFSRMATSTPALSEFDNYHKAKVSSLEEPSKEKSKTIKELVTMSSKLDSLEKGESFLREKIRAQKLKYNDKPDSLRQSNGEAFQKYLEDTTKNLIKAQPNLKANLVLHA

SEQ ID NO: 188 - protein, 138 aa, Gossypium barbadense
MIPQQMKLAFQSYIAFKSDSSPFSRMATSTPALSEFDNYHKAKVSSLEEPSKEKSKTIKELVTMSSKLDSLEKGESFLREKIRAQKLKYNDKPDSLRQSNGEAFQKYLEDTTKNLIKAQPNLKANLVLHAWSHPQFEK

SEQ ID NO: 189 - protein, 138 aa, Gossypium barbadense
WSHPQFEKMIPQQMKLAFQSYIAFKSDSSPFSRMATSTPALSEFDNYHKAKVSSLEEPSKEKSKTIKELVTMSSKLDSLEKGESFLREKIRAQKLKYNDKPDSLRQSNGEAFQKYLEDTTKNLIKAQPNLKANLVLHA

SEQ ID NO: 190 - protein, 140 aa, Gossypium barbadense
MIPQQMKLAFQSYIAFKSDSSPFSRMATSTPALSEFDNYHKAKVSSLEEPSKEKSKTIKELVTMSSKLDSLEKGESFLREKIRAQKLKYNDKPDSLRQSNGEAFQKYLEDTTKNLIKAQPNLKANLVLHAEQKLISEEDL

SEQ ID NO: 191 - protein, 140 aa, Gossypium barbadense
EQKLISEEDLMIPQQMKLAFQSYIAFKSDSSPFSRMATSTPALSEFDNYHKAKVSSLEEPSKEKSKTIKELVTMSSKLDSLEKGESFLREKIRAQKLKYNDKPDSLRQSNGEAFQKYLEDTTKNLIKAQPNLKANLVLHA

SEQ ID NO: 192 - DNA, 393 bp, Gossypium barbadense
  source 1..393: mol_type = other DNA
atgatccctcaacaaatgaaaaaaaaaaaacaatcttactttaaaatagcctcagactcatctgccgcccaacaaatggctaaatctaccaattatcatcctgctttatctgaatttgataaagttaaggtttgggaggagtcctccccaagtaaatcaaaaagcaagacgataaaggagttagttacaatgagcagtaagcttgattcattggagaaaggcgagtccttcttaagggaaaaaatccaagcccagaagctaaaatataatgacaagccggatagccttcgccagtccaatggtgaagcctttcaaaagtacctagaggacacaaccaagaacttgatcaaggcaatgccagcccaacaagctaacttggtccttcatgcctaa

SEQ ID NO: 193 - DNA, 390 bp, Gossypium barbadense
  source 1..390: mol_type = other DNA
cagcagatgatgattcctaaagaagcttttttcaagtctgattcccaatcatatatcgcctcgccctttagtcgtatgaaagcaagcactccagcgttattggagttcgactactatcataaggttaaagtctctgctcttgaagagccgtccaagtcaaaatcgaagaccataaaagaactcgtaacaatgagtagcaagctagattctctggagaaaggtgaatcctttttacgcgagaagattcaggcccaaaaattgaagtacaatgacaaacctgattcacttcgacagtcgaacggcgaagcattccaaaagtatctcgaggacacgactaaaaatctaatcaaggcgatgcccaacctggctaaaaatttagtgttgcacgcc

SEQ ID NO: 194 - DNA, 390 bp, Gossypium barbadense
  source 1..390: mol_type = other DNA
caacagatgatgattcctaaagaagcttttttcaagtctgattcccaatcatatatcgcctcgccctttagtcgtatgaaagcaagcactccagcgttattggagttcgactactatcataaggttaaagtctctgctcttgaagagccgtccaagtcaaaatcgaagaccataaaagaactcgtaacaatgagtagcaagctagattctctggagaaaggtgaatcctttttacgcgagaagattcaggcccaaaaattgaagtacaatgacaaacctgattcacttcgacagtcgaacggcgaagcattccaaaagtatctcgaggacacgactaaaaatctaatcaaggcgatgcccaacctggctaaaaatttagtgttgcacgcc

SEQ ID NO: 195 - DNA, 390 bp, Gossypium barbadense
  source 1..390: mol_type = other DNA
atgattcctcaacagatgaaagaagcttttcaatcttatatcgccttcaagtccgattcaatggcaaaatcgactagtccctttagccgtccagcgttatctgagttcgacaattaccataaggctaaagtttcctcattgtttgaaccgtcgaagagtaaaagcaagaccataaaagagcttgtcacaatgtcttccaagctcgattcactagaaaaaggtgagtcgttcctgcgcgaaaagattcaggcccaaaaattaaagtataacgacaaacctgatagtttgcgacagagcaatggcgaggcatttcaaaagtaccttgaagacacgactaaaaacctcatcaaggcgatgcccaatctaaaagctaacctggtattacacgcc

SEQ ID NO: 196 - DNA, 390 bp, Gossypium barbadense
  source 1..390: mol_type = other DNA
atgattcctcaacccatgaaagaagcttttcagtcttatatcgccttcaagtccgattcatcgccatttagtgttatggcaaaaagcactccggcgttatctgagttcgacaattaccataaggctaaagtctccgccttggaagagccttcaaagtcgaaaagtaagaccataaaagaacttgtaacaatgagctctaagctcgattccctagagaaaggtgaatcatttctgcgtgagaagattcaagcacagaaattaaagtataacgacaaacccgattcgttgcgccaaagtaatggcgaagcgttccagaagtaccttgaggacacgactaaaaacctcatcaaggctatgccaaatctaaaagccatgctggtgttacacgca

SEQ ID NO: 197 - DNA, 390 bp, Gossypium barbadense
  source 1..390: mol_type = other DNA
atgcctccccaagctatgaaattatttttccagtctgttattgccaagaaatccttgtcatcgccagtcagtagctctgcaacttccaccccggcgatctcaggttttgataatatgataaaggctaaagcctcgagtcttgaagagcctagcaaggaaaaatctaagacaattaaacaaatcgtaacgatgtcctcaaagctcatgtcgctagagaaaggcgaaagtcagctgcgtgtgaagttacgcatgcaaaaattgaagtataacaaaaagaaagacagccttcgacagtctaatcccgaggcattccaaaagtacctcgaagatactaccaaaaacgttataaagatgcaggtcaatcggaaagcgaacctagtactgcatgct

SEQ ID NO: 198 - DNA, 390 bp, Gossypium barbadense
  source 1..390: mol_type = other DNA
atgcctccccaacagatgaaattatttttccaatctgttattgcttttaagtccttgtcatcgccagtcagtcgtatggccactagcaccccggcaatctctggtttcgataatatgataaaagcgaaggcttcctcacttgaagagccttcgaaagaaaagagtaaaacaattaagcagatcgtaacgatgagctctaaactcatgtccctagagaagggcgaatcatttctgcgcgtgaaattacgaatgcaaaagttgaaatataacgacaagcccgattcgcttcggcagagtaatggagaggccttccaaaaatacctcgaagacactaccaagaacgttataaaaatgcaggtcaatagaaaggcaaacctagtactgcatgcg

SEQ ID NO: 199 - DNA, 390 bp, Gossypium barbadense
  source 1..390: mol_type = other DNA
atgattcctcaattaatgaaaggtatgtttcagtcttatatcatgttcacttccgatgactcacccttttcgcgtatggctgttagtaccccagccttggtcgaattcgataattacaagaaagcaaaggtaagctctcttgtgtccccgtcaaaatcgaagagtaaaacaataaaggaggttgtcacgcgcagctctaaactcgactccctagaaaagggcgagtcactgttacgagaaaaacggcaatcgcagaagttgaaatataacgataagcctgacagtcttagacaaagcaatggagaggcgtttcagaaatacctcgaagatactaccaagaacctaatgaaagctatgagggtactgaaggccaatttagtgttgcatgca

SEQ ID NO: 200 - DNA, 432 bp, Gossypium barbadense
  source 1..432: mol_type = other DNA
atgattcctcaattaatgaaaaagatgttttaacagtcttatatcatgttcaaatccgattcatagtcgccctttagtcgtatggctgttagcacttgaccagccttggtcgaattcgacaattacaagtaaaaagcaaaggtatcttcccttgagtcaccgtagtcgaaaagtaagagcaaaaccataaaggaatgagtggttacacgctcttccaaactcgattcataactagagaagggtgaatcgtttctgcgagagtagaaacggcaaagtcagaagttaaaatataactgagacaagcctgatagcttgagacaatctaattaaggcgaagcgttccagaaataccttgaggactagacgactaagaacctcatgaaagctatgaggtgagtcctaaaggccaatctggtattacatgcataatag

SEQ ID NO: 201 - DNA, 435 bp, Gossypium barbadense
  source 1..435: mol_type = other DNA
atgattcctcaacagatgaaattagctttttaacaatcttatatcgccttcaagtccgattcatagtcgccctttagtcgtatggcaactagcacctgaccagcgttgtctgaattcgacaattaccattaaaaagctaaggtttcctcacttgaggaaccgtagtcgaaagagaagagtaaaacaataaaggaatgactcgtcacgatgagctctaaactagattcctaactggagaagggtgaatcatttttacgcgagtagaaaattcgagcccagaagttgaaatataactgagacaagcctgattcgcttcggcaaagtaattaaggcgaagcattccagaaatacctcgaggactagactaccaagaacctaatcaaagcgcaaccctgataaaatctgaaggctaacttagtattgcacgcctagtga

SEQ ID NO: 202 - DNA, 405 bp, Gossypium barbadense
  source 1..405: mol_type = other DNA
atgattcctcaacagatgaaagaagcttttcaatcttatatcgccttcaagtccgattcatcgccctttagtcgtatggcaaaaagcactccagcgttatctgagttcgacaattaccataaggctaaagtttcctcattggaagagccgtcgaagagtaaaagccctaccataaaggaacttgtcacaccctcttccaaactcgattcactagagaagggtgaatcgtttctgcgcgagaaaattcaggcccaaaagaaaaagtataacgacaaaccagcaagtttaccgcagagcaatggcgaagcgttccaaaagtacttggaggatacgactaaaaaccttatcaaggctatgcctaatctcaaagccaacctagtactgcacgcacgacggagaaggcgt

SEQ ID NO: 203 - DNA, 405 bp, Gossypium barbadense
  source 1..405: mol_type = other DNA
cgtcgccgacggagaatgattcctcaacagatgaaagaagcttttcaatcttatatcgccttcaagtccgattcatcgccctttagtaggatggcaaaaagcactccagcgttatctgagttcgacaattaccataaggctaaagtttcctcattggaagagccgtcgaagagtaaaagccctaccataaaggaacttgtcacaccctcttccaaactcgattcactagagaagggtgaatcgtttctgcgtgagaaaattcaggcccaaaagaaaaagtataacgacaaaccagcaagtttaccgcagagcaatggcgaagcgttccaaaagtacttggaggatacgactaaaaaccttatcaaggctatgcctaatctcaaagccaacctagtactgcacgca

SEQ ID NO: 204 - DNA, 408 bp, Gossypium barbadense
  source 1..408: mol_type = other DNA
atgattcctcaacagatgaaagaagcttttcaatcttatatcgccttcaagtccgattcatcgccctttagtcgtatggcaaaaagcactccagcgttatctgagttcgacaattaccataaggctaaagtttcctcattggaagagccgtcgaagagtaaaagccctaccataaaggaacttgtcacaccctcttccaaactcgattcactagagaagggtgaatcgtttctgcgcgagaaaattcaggcccaaaagaaaaagtataacgacaaaccagcaagtttaccgcagagcaatggcgaagcgttccaaaagtacttggaggatacgactaaaaaccttatcaaggctatgcctaatctcaaagccaacctagtactgcacgcacgacggagaaggcgtcgc

SEQ ID NO: 205 - DNA, 408 bp, Gossypium barbadense
  source 1..408: mol_type = other DNA
cgtcgccgacggagaaggatgattcctcaacagatgaaagaagcttttcaatcttatatcgccttcaagtccgattcatcgccctttagtcgtatggcaaaaagcactccagcgttatctgagttcgacaattaccataaggctaaagtttcctcattggaagagccgtcgaagagtaaaagccctaccataaaggaacttgtcacaccctcttccaaactcgattcactagagaagggtgaatcgtttctgcgcgagaaaattcaggcccaaaagaaaaagtataacgacaaaccagcaagtttaccgcagagcaatggcgaagcgttccaaaagtacttggaggatacgactaaaaaccttatcaaggctatgcctaatctcaaagccaacctagtactgcacgca

SEQ ID NO: 206 - DNA, 396 bp, Gossypium barbadense
  source 1..396: mol_type = other DNA
atgattcctcaacagatgaaagaagcttttcaatcttatatcgccttcaagtccgattcatcgccctttagtcgtatggcaaaaagcactccagcgttatctgagttcgacaattaccataaggctaaagtttcctcattggaagagccgtcgaagagtaaaagccctaccataaaggaacttgtcacaccctcttccaaactcgattcactagagaagggtgaatcgtttctgcgcgagaaaattcaggcccaaaagaaaaagtataacgacaaaccagcaagtttaccgcagagcaatggcgaagcgttccaaaagtacttggaggatacgactaaaaaccttatcaaggctatgcctaatctcaaagccaacctagtactgcacgcacatcac

SEQ ID NO: 207 - DNA, 420 bp, Gossypium barbadense
  source 1..420: mol_type = other DNA
catcaccatcaccatcaccatcaccatcacatgattcctcaacagatgaaagaagcttttcaatcttatatcgccttcaagtccgattcatcgccctttagtcgtatggcaaaaagcactccagcgttatctgagttcgacaattaccataaggctaaagtttcctcattggaagagccgtcgaagagtaaaagccctaccataaaggaacttgtcacaccctcttccaaactcgattcactagagaagggtgaatcgtttctgcgcgagaaaattcaggcccaaaagaaaaagtataacgacaaaccagcaagtttaccgcagagcaatggcgaagcgttccaaaagtacttggaggatacgactaaaaaccttatcaaggctatgcctaatctcaaagccaacctagtactgcacgca

SEQ ID NO: 208 - DNA, 402 bp, Gossypium barbadense
  source 1..402: mol_type = other DNA
atgattcctcaacagatgaaagaagcttttcaatcttatatcgccttcaagtccgattcatcgccctttagtcgtatggcaaaaagcactccagcgttatctgagttcgacaattaccataaggctaaagtttcctcattggaagagccgtcgaagagtaaaagccctaccataaaggaacttgtcacaccctcttccaaactcgattcactagagaagggtgaatcgtttctgcgcgagaaaattcaggcccaaaagaaaaagtataacgacaaaccagcaagtttaccgcagagcaatggcgaagcgttccaaaagtacttggaggatacgactaaaaaccttatcaaggctatgcctaatctcaaagccaacctagtactgcacgcacatcaccatcac

SEQ ID NO: 209 - DNA, 396 bp, Gossypium barbadense
  source 1..396: mol_type = other DNA
catcacatgattcctcaacagatgaaagaagcttttcaatcttatatcgccttcaagtccgattcatcgccctttagtcgtatggcaaaaagcactccagcgttatctgagttcgacaattaccataaggctaaagtttcctcattggaagagccgtcgaagagtaaaagccctaccataaaggaacttgtcacaccctcttccaaactcgattcactagagaagggtgaatcgtttctgcgcgagaaaattcaggcccaaaagaaaaagtataacgacaaaccagcaagtttaccgcagagcaatggcgaagcgttccaaaagtacttggaggatacgactaaaaaccttatcaaggctatgcctaatctcaaagccaacctagtactgcacgca

SEQ ID NO: 210 - DNA, 411 bp, Gossypium barbadense
  source 1..411: mol_type = other DNA
catcaccatcaccatcaccatatgattcctcaacagatgaaagaagcttttcaatcttatatcgccttcaagtccgattcatcgccctttagtcgtatggcaaaaagcactccagcgttatctgagttcgacaattaccacaaggctaaagtttcctcattggaagagccgtcgaagagtaaaagccctaccataaaggaacttgtcacaccctcttccaaactcgattcactagagaagggtgaatcgtttctgcgcgagaaaattcaggcccaaaagaaaaagtataacgacaaaccagcaagtttaccgcagagcaatggcgaagcgttccaaaagtacttggaggatacgactaaaaaccttatcaaggctatgcctaatctcaaagccaacctagtactgcatgca

SEQ ID NO: 211 - DNA, 420 bp, Gossypium barbadense
  source 1..420: mol_type = other DNA
atgattcctcaacagatgaaagaagcttttcaatcttatatcgccttcaagtccgattcatcgccctttagtcgtatggcaaaaagcactccagcgttatctgagttcgacaattaccataaggctaaagtttcctcattggaagagccgtcgaagagtaaaagccctaccataaaggaacttgtcacaccctcttccaaactcgattcactagagaagggtgaatcgtttctgcgcgagaaaattcaggcccaaaagaaaaagtataacgacaaaccagcaagtttaccgcagagcaatggcgaagcgttccaaaagtacttggaggatacgactaaaaaccttatcaaggctatgcctaatctcaaagccaacctagtactgcacgcacatcaccatcaccatcaccatcaccatcac

SEQ ID NO: 212 - DNA, 414 bp, Gossypium barbadense
  source 1..414: mol_type = other DNA
atgattcctcaacagatgaaagaagcttttcaatcttatatcgccttcaagtccgattcatcgccctttagtcgtatggcaaaaagcactccagcgttatctgagttcgacaattaccataaggctaaagtttcctcattggaagagccgtcgaagagtaaaagccctaccataaaggaacttgtcacaccctcttccaaactcgattcactagagaagggtgaatcgtttctgcgcgagaaaattcaggcccaaaagaaaaagtataacgacaaaccagcaagtttaccgcagagcaatggcgaagcgttccaaaagtacttggaggatacgactaaaaaccttatcaaggctatgcctaatctcaaagccaacctagtactgcacgcagactataaggatgacgatgacaaa

SEQ ID NO: 213 - DNA, 414 bp, Gossypium barbadense
  source 1..414: mol_type = other DNA
gattataaagacgatgacgataagatgattcctcaacagatgaaagaagcttttcaatcttacatcgccttcaagtccgactcatcgccctttagtcgtatggcaaaaagcactccagcgttatctgagttcgataattatcataaggctaaagtttcctcattggaagagccgtcgaagagtaaaagccctaccataaaggaacttgtcacaccctcttccaaactcgactcactagagaagggtgaatcgtttctgcgcgagaaaattcaggcccaaaagaaaaagtacaacgataaaccagcaagtttaccgcagagcaatggcgaagcgttccaaaagtatttggaggacacgactaaaaaccttatcaaggctatgcctaatctcaaagccaacctagtactgcacgca

SEQ ID NO: 214 - DNA, 414 bp, Gossypium barbadense
  source 1..414: mol_type = other DNA
atgattcctcaacagatgaaagaagcttttcaatcttatatcgccttcaagtccgattcatcgccctttagtcgtatggcaaaaagcactccagcgttatctgagttcgacaattaccataaggctaaagtttcctcattggaagagccgtcgaagagtaaaagccctaccataaaggaacttgtcacaccctcttccaaactcgattcactagagaagggtgaatcgtttctgcgcgagaaaattcaggcccaaaagaaaaagtataacgacaaaccagcaagtttaccgcagagcaatggcgaagcgttccaaaagtacttggaggatacgactaaaaaccttatcaaggctatgcctaatctcaaagccaacctagtactgcacgcatggtctcatccccagtttgaaaag

SEQ ID NO: 215 - DNA, 414 bp, Gossypium barbadense
  source 1..414: mol_type = other DNA
tggtctcatcctcaatttgaaaaaatgattccccagcaaatgaaggaggctttccagtcctatatcgcctttaaatcagattcgagtccattcagccgtatggcaaagtctactccggcgttatccgaatttgacaattaccacaaagctaaggtttcatcgttggaggaacctagtaaaagcaagtctcccaccataaaagagcttgtcacaccatcctcaaagctcgattcgctagaaaaaggtgagagtttcctgcgcgaaaagattcaagcccagaaaaagaaatataacgacaagccggcaagcttacctcaatctaatggcgaggcgtttcagaaatacttggaagatacgactaagaaccttatcaaagctatgcccaatctcaaggccaacctagtactgcatgca

SEQ ID NO: 216 - DNA, 420 bp, Gossypium barbadense
  source 1..420: mol_type = other DNA
atgattcctcaacagatgaaagaagcttttcaatcttatatcgccttcaagtccgattcatcgccctttagtcgtatggcaaaaagcactccagcgttatctgagttcgacaattaccataaggctaaagtttcctcattggaagagccgtcgaagagtaaaagccctaccataaaggaacttgtcacaccctcttccaaactcgattcactagagaagggtgaatcgtttctgcgcgagaaaattcaggcccaaaagaaaaagtataacgacaaaccagcaagtttaccgcagagcaatggcgaagcgttccaaaagtacttggaggatacgactaaaaaccttatcaaggctatgcctaatctcaaagccaacctagtactgcacgcagaacagaagttaatatctgaggaagacttg

SEQ ID NO: 217 - DNA, 420 bp, Gossypium barbadense
  source 1..420: mol_type = other DNA
gaacaaaaattaatttctgaggaagatttgatgatccctcagcaaatgaaggaggcttttcagtcctatatagccttcaaatcagactcgagtccctttagccgtatggcaaagtctactccagcgctttccgaattcgataattaccataaagctaaggtttcatcgctcgaggaaccgagtaaaagcaagtctcctaccattaaagagctagtcacaccctcctcaaagctggactcgttagaaaaaggtgagagttttttgcgcgaaaagatccaagcccagaaaaagaaatataacgataagccagcaagccttccgcaatctaatggcgaggcgttccagaaatacctcgaagacacgactaagaacctaataaaagctatgcctaatctgaaggccaacttagtattgcacgca